European Patent Application EP 4 796 562 A1, published August 26, 2026. Title: 一种靶向δ样配体3的CAR及应用. Applicant: 上海先博生物科技有限公司. Application CN. The sequence listing filed with the application follows.

SEQUENCE LISTING (106 sequences)

SEQ ID NO: 1 - protein, 122 aa, Synthetic construct
EVQLQQSGPVLVKPGASVKMSCKASGYTFTDYYMNWVKRSHGKSLEWIGIINPYNGGTSYNQKFRGKATLTVDKSSNTAYMELNSLTSEDSAVYYCSRYDYDYDVEGAMDYWGQGTSVTVSS

SEQ ID NO: 2 - protein, 107 aa, Synthetic construct
DIVMTQSQKFMSTSVGDRVSITCKASQNVGTAVAWYQQKPGQSPKLLIFSASIRYTGVPDRFTGSGSGTDFTLTISNMQSEDLADYFCQQYSSSPYTFGGGTKLEIK

SEQ ID NO: 3 - protein, 118 aa, Synthetic construct
EVQLQQSGTVLARPGASVKMSCKTSGYTFTSYWMHWVKQSPGQGLEWIGTIYPGNSDTRYNQKFKDKAYVTAVTSASTAYMELSSLTNEESAVYYCTRSYDYGDLDYWGQGTTLTVSS

SEQ ID NO: 4 - protein, 107 aa, Synthetic construct
DIVMTQSPATLSVTPGDRVSLSCRASQTISDYLHWYQQRSHESPRLLIKYASQSISGIPSRFSGSGSGSDFTLSINSVEPEDVGVYYCQNGHSFPLTFGAGTKLELK

SEQ ID NO: 5 - protein, 119 aa, Synthetic construct
QVQLQQSGAELVKPGASVRISCKASGYAFSNYWINWVKQRPGKGLEWIGQINPGDGDTIYNGKFKGKATLTADKSSSTAYMQLSSLTSEDSAVYFCEREGRNYGDFAYWGQGTTLTVSS

SEQ ID NO: 6 - protein, 111 aa, Synthetic construct
DIVLTQSPASLAVSLGQRATISCRASKSVSTSGFSYMHWYQQKPGQPPKLLIYLASNLESGVPARFSGSGSGTDFTLNIHPVEEEDAATYYCQHSRELPFTFGSGTKLEIK

SEQ ID NO: 7 - protein, 5 aa, Synthetic construct
DYYMN

SEQ ID NO: 8 - protein, 17 aa, Synthetic construct
IINPYNGGTSYNQKFRG

SEQ ID NO: 9 - protein, 13 aa, Synthetic construct
YDYDYDVEGAMDY

SEQ ID NO: 10 - protein, 11 aa, Synthetic construct
KASQNVGTAVA

SEQ ID NO: 11 - protein, 7 aa, Synthetic construct
SASIRYT

SEQ ID NO: 12 - protein, 9 aa, Synthetic construct
QQYSSSPYT

SEQ ID NO: 13 - protein, 5 aa, Synthetic construct
SYWMH

SEQ ID NO: 14 - protein, 17 aa, Synthetic construct
TIYPGNSDTRYNQKFKD

SEQ ID NO: 15 - protein, 9 aa, Synthetic construct
SYDYGDLDY

SEQ ID NO: 16 - protein, 11 aa, Synthetic construct
RASQTISDYLH

SEQ ID NO: 17 - protein, 7 aa, Synthetic construct
YASQSIS

SEQ ID NO: 18 - protein, 9 aa, Synthetic construct
QNGHSFPLT

SEQ ID NO: 19 - protein, 5 aa, Synthetic construct
NYWIN

SEQ ID NO: 20 - protein, 17 aa, Synthetic construct
QINPGDGDTIYNGKFKG

SEQ ID NO: 21 - protein, 10 aa, Synthetic construct
EGRNYGDFAY

SEQ ID NO: 22 - protein, 15 aa, Synthetic construct
RASKSVSTSGFSYMH

SEQ ID NO: 23 - protein, 7 aa, Synthetic construct
LASNLES

SEQ ID NO: 24 - protein, 9 aa, Synthetic construct
QHSRELPFT

SEQ ID NO: 25 - protein, 8 aa, Synthetic construct
GYTFTDYY

SEQ ID NO: 26 - protein, 8 aa, Synthetic construct
INPYNGGT

SEQ ID NO: 27 - protein, 15 aa, Synthetic construct
SRYDYDYDVEGAMDY

SEQ ID NO: 28 - protein, 6 aa, Synthetic construct
QNVGTA

SEQ ID NO: 29 - skipped

SEQ ID NO: 30 - protein, 9 aa, Synthetic construct
QQYSSSPYT

SEQ ID NO: 31 - protein, 8 aa, Synthetic construct
GYTFTSYW

SEQ ID NO: 32 - protein, 8 aa, Synthetic construct
IYPGNSDT

SEQ ID NO: 33 - protein, 11 aa, Synthetic construct
TRSYDYGDLDY

SEQ ID NO: 34 - protein, 6 aa, Synthetic construct
QTISDY

SEQ ID NO: 35 - skipped

SEQ ID NO: 36 - protein, 9 aa, Synthetic construct
QNGHSFPLT

SEQ ID NO: 37 - protein, 8 aa, Synthetic construct
GYAFSNYW

SEQ ID NO: 38 - protein, 8 aa, Synthetic construct
INPGDGDT

SEQ ID NO: 39 - protein, 12 aa, Synthetic construct
EREGRNYGDFAY

SEQ ID NO: 40 - protein, 10 aa, Synthetic construct
KSVSTSGFSY

SEQ ID NO: 41 - skipped

SEQ ID NO: 42 - protein, 9 aa, Synthetic construct
QHSRELPFT

SEQ ID NO: 43 - protein, 7 aa, Synthetic construct
GYTFTDY

SEQ ID NO: 44 - protein, 6 aa, Synthetic construct
NPYNGG

SEQ ID NO: 45 - protein, 13 aa, Synthetic construct
YDYDYDVEGAMDY

SEQ ID NO: 46 - protein, 11 aa, Synthetic construct
KASQNVGTAVA

SEQ ID NO: 47 - protein, 7 aa, Synthetic construct
SASIRYT

SEQ ID NO: 48 - protein, 9 aa, Synthetic construct
QQYSSSPYT

SEQ ID NO: 49 - protein, 7 aa, Synthetic construct
GYTFTSY

SEQ ID NO: 50 - protein, 6 aa, Synthetic construct
YPGNSD

SEQ ID NO: 51 - protein, 9 aa, Synthetic construct
SYDYGDLDY

SEQ ID NO: 52 - protein, 11 aa, Synthetic construct
RASQTISDYLH

SEQ ID NO: 53 - protein, 7 aa, Synthetic construct
YASQSIS

SEQ ID NO: 54 - protein, 9 aa, Synthetic construct
QNGHSFPLT

SEQ ID NO: 55 - protein, 7 aa, Synthetic construct
GYAFSNY

SEQ ID NO: 56 - protein, 6 aa, Synthetic construct
NPGDGD

SEQ ID NO: 57 - protein, 10 aa, Synthetic construct
EGRNYGDFAY

SEQ ID NO: 58 - protein, 15 aa, Synthetic construct
RASKSVSTSGFSYMH

SEQ ID NO: 59 - protein, 7 aa, Synthetic construct
LASNLES

SEQ ID NO: 60 - protein, 9 aa, Synthetic construct
QHSRELPFT

SEQ ID NO: 61 - protein, 21 aa, Synthetic construct
MALPVTALLLPLALLLHAARP

SEQ ID NO: 62 - protein, 45 aa, Synthetic construct
TTTPAPRPPTPAPTIASQPLSLRPEACRPAAGGAVHTRGLDFACD

SEQ ID NO: 63 - protein, 39 aa, Synthetic construct
IEVMYPPPYLDNEKSNGTIIHVKGKHLCPSPLFPGPSKP

SEQ ID NO: 64 - protein, 24 aa, Synthetic construct
IYIWAPLAGTCGVLLLSLVITLYC

SEQ ID NO: 65 - protein, 27 aa, Synthetic construct
FWVLVVVGGVLACYSLLVTVAFIIFWV

SEQ ID NO: 66 - protein, 42 aa, Synthetic construct
KRGRKKLLYIFKQPFMRPVQTTQEEDGCSCRFPEEEEGGCEL

SEQ ID NO: 67 - protein, 41 aa, Synthetic construct
RSKRSRLLHSDYMNMTPRRPGPTRKHYQPYAPPRDFAAYRS

SEQ ID NO: 68 - protein, 112 aa, Synthetic construct
RVKFSRSADAPAYQQGQNQLYNELNLGRREEYDVLDKRRGRDPEMGGKPRRKNPQEGLYNELQKDKMAEAYSEIGMKGERRRGKGHDGLYQGLSTATKDTYDALHMQALPPR

SEQ ID NO: 69 - protein, 18 aa, Synthetic construct
EGRGSLLTCGDVEENPGP

SEQ ID NO: 70 - protein, 15 aa, Synthetic construct
GGGGSGGGGSGGGGS

SEQ ID NO: 71 - protein, 20 aa, Synthetic construct
GGGGSGGGGSGGGGSGGGGS

SEQ ID NO: 72 - protein, 244 aa, Synthetic construct
DIVMTQSQKFMSTSVGDRVSITCKASQNVGTAVAWYQQKPGQSPKLLIFSASIRYTGVPDRFTGSGSGTDFTLTISNMQSEDLADYFCQQYSSSPYTFGGGTKLEIKGGGGSGGGGSGGGGSEVQLQQSGPVLVKPGASVKMSCKASGYTFTDYYMNWVKRSHGKSLEWIGIINPYNGGTSYNQKFRGKATLTVDKSSNTAYMELNSLTSEDSAVYYCSRYDYDYDVEGAMDYWGQGTSVTVSS

SEQ ID NO: 73 - protein, 240 aa, Synthetic construct
DIVMTQSPATLSVTPGDRVSLSCRASQTISDYLHWYQQRSHESPRLLIKYASQSISGIPSRFSGSGSGSDFTLSINSVEPEDVGVYYCQNGHSFPLTFGAGTKLELKGGGGSGGGGSGGGGSEVQLQQSGTVLARPGASVKMSCKTSGYTFTSYWMHWVKQSPGQGLEWIGTIYPGNSDTRYNQKFKDKAYVTAVTSASTAYMELSSLTNEESAVYYCTRSYDYGDLDYWGQGTTLTVSS

SEQ ID NO: 74 - protein, 245 aa, Synthetic construct
DIVLTQSPASLAVSLGQRATISCRASKSVSTSGFSYMHWYQQKPGQPPKLLIYLASNLESGVPARFSGSGSGTDFTLNIHPVEEEDAATYYCQHSRELPFTFGSGTKLEIKGGGGSGGGGSGGGGSQVQLQQSGAELVKPGASVRISCKASGYAFSNYWINWVKQRPGKGLEWIGQINPGDGDTIYNGKFKGKATLTADKSSSTAYMQLSSLTSEDSAVYFCEREGRNYGDFAYWGQGTTLTVSS

SEQ ID NO: 75 - protein, 492 aa, Synthetic construct
MALPVTALLLPLALLLHAARPQLQLQESGPGLVKPSETLSLTCTVSGGSISSSSYYWGWIRQPPGKGLEWIGSIYYSGNIYHNPSLKSRVSISVDTSKNQFSLRLSSVTAADTAVYYCAREIIVGATHFDYWGQGTLVTVSSGGGGSGGGGSGGGGSGGGGSAIQMTQSPSSLSASVGDRVTITCRASQGIRNDLGWYQQKPGKAPELLIYAASSLQSGVPSRFSGSGSGTDFTLTISSLQPEDFATYYCLQDYNYPLTFGPGTKVDIKTTTPAPRPPTPAPTIASQPLSLRPEACRPAAGGAVHTRGLDFACDIYIWAPLAGTCGVLLLSLVITLYCKRGRKKLLYIFKQPFMRPVQTTQEEDGCSCRFPEEEEGGCELRVKFSRSADAPAYQQGQNQLYNELNLGRREEYDVLDKRRGRDPEMGGKPRRKNPQEGLYNELQKDKMAEAYSEIGMKGERRRGKGHDGLYQGLSTATKDTYDALHMQALPPR

SEQ ID NO: 76 - protein, 509 aa, Synthetic construct
MALPVTALLLPLALLLHAARPQVQLVESGGGVVQPGGSLRLSCAASFSGYGVSTMAWFRQAPGKGLEGVAAITVGSGNTYYADSVKGRFTISRDNSKNTVYLQMNSLRAEDTAMYYCAVGYLSGGSWDVPGRYNYWGQGTLVTVSSGGGGSGGGGSGGGGSEVQLVESGGGLVQPGGSLRLSCAASGNTYSSNYMGWFRQAPGKGLEEVAVIYTRGGHTYYVDSVRGRFTISQDNAKNSLYLQMNSLRAEDTAVYYCAASSRHRLGLNNPRDYDYWGQGTLVTVSSTTTPAPRPPTPAPTIASQPLSLRPEACRPAAGGAVHTRGLDFACDIYIWAPLAGTCGVLLLSLVITLYCKRGRKKLLYIFKQPFMRPVQTTQEEDGCSCRFPEEEEGGCELRVKFSRSADAPAYKQGQNQLYNELNLGRREEYDVLDKRRGRDPEMGGKPRRKNPQEGLYNELQKDKMAEAYSEIGMKGERRRGKGHDGLYQGLSTATKDTYDALHMQALPPR

SEQ ID NO: 77 - protein, 488 aa, Synthetic construct
MALPVTALLLPLALLLHAARPDIVMTQSQKFMSTSVGDRVSITCKASQNVGTAVAWYQQKPGQSPKLLIFSASIRYTGVPDRFTGSGSGTDFTLTISNMQSEDLADYFCQQYSSSPYTFGGGTKLEIKGGGGSGGGGSGGGGSEVQLQQSGPVLVKPGASVKMSCKASGYTFTDYYMNWVKRSHGKSLEWIGIINPYNGGTSYNQKFRGKATLTVDKSSNTAYMELNSLTSEDSAVYYCSRYDYDYDVEGAMDYWGQGTSVTVSSTTTPAPRPPTPAPTIASQPLSLRPEACRPAAGGAVHTRGLDFACDIYIWAPLAGTCGVLLLSLVITLYCKRGRKKLLYIFKQPFMRPVQTTQEEDGCSCRFPEEEEGGCELRVKFSRSADAPAYQQGQNQLYNELNLGRREEYDVLDKRRGRDPEMGGKPRRKNPQEGLYNELQKDKMAEAYSEIGMKGERRRGKGHDGLYQGLSTATKDTYDALHMQALPPR

SEQ ID NO: 78 - protein, 484 aa, Synthetic construct
MALPVTALLLPLALLLHAARPDIVMTQSPATLSVTPGDRVSLSCRASQTISDYLHWYQQRSHESPRLLIKYASQSISGIPSRFSGSGSGSDFTLSINSVEPEDVGVYYCQNGHSFPLTFGAGTKLELKGGGGSGGGGSGGGGSEVQLQQSGTVLARPGASVKMSCKTSGYTFTSYWMHWVKQSPGQGLEWIGTIYPGNSDTRYNQKFKDKAYVTAVTSASTAYMELSSLTNEESAVYYCTRSYDYGDLDYWGQGTTLTVSSTTTPAPRPPTPAPTIASQPLSLRPEACRPAAGGAVHTRGLDFACDIYIWAPLAGTCGVLLLSLVITLYCKRGRKKLLYIFKQPFMRPVQTTQEEDGCSCRFPEEEEGGCELRVKFSRSADAPAYQQGQNQLYNELNLGRREEYDVLDKRRGRDPEMGGKPRRKNPQEGLYNELQKDKMAEAYSEIGMKGERRRGKGHDGLYQGLSTATKDTYDALHMQALPPR

SEQ ID NO: 79 - protein, 489 aa, Synthetic construct
MALPVTALLLPLALLLHAARPDIVLTQSPASLAVSLGQRATISCRASKSVSTSGFSYMHWYQQKPGQPPKLLIYLASNLESGVPARFSGSGSGTDFTLNIHPVEEEDAATYYCQHSRELPFTFGSGTKLEIKGGGGSGGGGSGGGGSQVQLQQSGAELVKPGASVRISCKASGYAFSNYWINWVKQRPGKGLEWIGQINPGDGDTIYNGKFKGKATLTADKSSSTAYMQLSSLTSEDSAVYFCEREGRNYGDFAYWGQGTTLTVSSTTTPAPRPPTPAPTIASQPLSLRPEACRPAAGGAVHTRGLDFACDIYIWAPLAGTCGVLLLSLVITLYCKRGRKKLLYIFKQPFMRPVQTTQEEDGCSCRFPEEEEGGCELRVKFSRSADAPAYQQGQNQLYNELNLGRREEYDVLDKRRGRDPEMGGKPRRKNPQEGLYNELQKDKMAEAYSEIGMKGERRRGKGHDGLYQGLSTATKDTYDALHMQALPPR

SEQ ID NO: 80 - protein, 729 aa, Synthetic construct
MALPVTALLLPLALLLHAARPQVQLVESGGGVVQPGGSLRLSCAASFSGYGVSTMAWFRQAPGKGLEGVAAITVGSGNTYYADSVKGRFTISRDNSKNTVYLQMNSLRAEDTAMYYCAVGYLSGGSWDVPGRYNYWGQGTLVTVSSGGGGSGGGGSGGGGSEVQLVESGGGLVQPGGSLRLSCAASGNTYSSNYMGWFRQAPGKGLEEVAVIYTRGGHTYYVDSVRGRFTISQDNAKNSLYLQMNSLRAEDTAVYYCAASSRHRLGLNNPRDYDYWGQGTLVTVSSTTTPAPRPPTPAPTIASQPLSLRPEACRPAAGGAVHTRGLDFACDIYIWAPLAGTCGVLLLSLVITLYCKRGRKKLLYIFKQPFMRPVQTTQEEDGCSCRFPEEEEGGCELRVKFSRSADAPAYKQGQNQLYNELNLGRREEYDVLDKRRGRDPEMGGKPRRKNPQEGLYNELQKDKMAEAYSEIGMKGERRRGKGHDGLYQGLSTATKDTYDALHMQALPPRGSGEGRGSLLTCGDVEENPGPMGRGLLRGLWPLHIVLWTRIASTIPPHVQKSVNNDMIVTDNNGAVKFPQLCKFCDVRFSTCDNQKSCMSNCSITSICEKPQEVCVAVWRKNDENITLETVCHDPKLPYHDFILEDAASPKCIMKEKKKPGETFFMCSCSSDECNDNIIFSEEYNTSNPDLLLVIFQVTGISLLPPLGVAISVIIIFYCYRVNRQQKLSS

SEQ ID NO: 81 - protein, 107 aa, Synthetic construct
DIQMTQSPSSLSASVGDRVTITCKASQNVGTAVAWYQQKPGKSPKLLIFSASIRYTGVPSRFSGSGSGTDFTLTISSLQPEDFATYYCQQYSSSPYTFGGGTKVEIK

SEQ ID NO: 82 - protein, 107 aa, Synthetic construct
DIVMTQSPDSLAVSLGERATINCKASQNVGTAVAWYQQKPGQSPKLLIFSASIRYTGVPDRFSGSGSGTDFTLTISSLQAEDVAVYYCQQYSSSPYTFGGGTKVEIK

SEQ ID NO: 83 - protein, 122 aa, Synthetic construct
EVQLVQSGAEVKKPGASVKVSCKASGYTFTDYYMNWVRQAPGQRLEWMGIINPYNSGTSYNQKFRGRVTLTVDKSASTAYMELSSLRSEDTAVYYCSRYDYDYDVEGAMDYWGQGTTVTVSS

SEQ ID NO: 84 - protein, 122 aa, Synthetic construct
EVQLVQSGAEVKKPGASVKVSCKASGYTFTDYYMNWVRRAPGQRLEWMGIINPYNGGTSYNQKFRGRVTITVDKSASTAYMELSSLRSEDTAVYYCSRYDYDYDVEGAMDYWGQGTTVTVSS

SEQ ID NO: 85 - protein, 107 aa, Synthetic construct
DIVMTQSPLSLPVTPGEPASISCRASQTISDYLHWYLQKPGQSPQLLIKYASQSISGVPDRFSGSGSGSDFTLKISRVEAEDVGVYYCQQGHSFPLTFGQGTKLEIK

SEQ ID NO: 86 - protein, 107 aa, Synthetic construct
DIVMTQSPLSLPVTPGEPASISCRASQTISDYLHWYLQKPGQSPRLLIKYASQSISGVPDRFSGSGSGTDFTLKISRVEAEDVGVYYCQNGHSFPLTFGQGTKLEIK

SEQ ID NO: 87 - protein, 118 aa, Synthetic construct
EVQLVQSGAEVKKPGASVKVSCKASGYTFTSYWMHWVRQAPGQRLEWMGTIYPGNSDTRYNQKFKDRVTITADTSASTAYMELSSLRSEDTAVYYCTRSYDYGDLDYWGQGTTVTVSS

SEQ ID NO: 88 - protein, 9 aa, Synthetic construct
QQGHSFPLT

SEQ ID NO: 89 - protein, 111 aa, Synthetic construct
EIVLTQSPATLSLSPGERATLSCRASKSVSTSGFSYMHWYQQKPGQPPRLLIYLASNLESGIPARFSGSGSGTDFTLTISSLEPEDFAVYYCQHSRELPFTFGQGTKLEIK

SEQ ID NO: 90 - protein, 119 aa, Synthetic construct
EVQLVQSGAEVKKPGSSVKVSCKASGYAFSNYWINWVRQAPGQGLEWMGQINPGDGDTIYNSKFKGRVTITADKSTSTAYMELSSLRSEDTAVYYCEREGRNYGDFAYWGQGTTVTVSS

SEQ ID NO: 91 - protein, 17 aa, Synthetic construct
QINPGDGDTIYNSKFKG

SEQ ID NO: 92 - protein, 488 aa, Synthetic construct
MALPVTALLLPLALLLHAARPDIQMTQSPSSLSASVGDRVTITCKASQNVGTAVAWYQQKPGKSPKLLIFSASIRYTGVPSRFSGSGSGTDFTLTISSLQPEDFATYYCQQYSSSPYTFGGGTKVEIKGGGGSGGGGSGGGGSEVQLVQSGAEVKKPGASVKVSCKASGYTFTDYYMNWVRQAPGQRLEWMGIINPYNSGTSYNQKFRGRVTLTVDKSASTAYMELSSLRSEDTAVYYCSRYDYDYDVEGAMDYWGQGTTVTVSSTTTPAPRPPTPAPTIASQPLSLRPEACRPAAGGAVHTRGLDFACDIYIWAPLAGTCGVLLLSLVITLYCKRGRKKLLYIFKQPFMRPVQTTQEEDGCSCRFPEEEEGGCELRVKFSRSADAPAYQQGQNQLYNELNLGRREEYDVLDKRRGRDPEMGGKPRRKNPQEGLYNELQKDKMAEAYSEIGMKGERRRGKGHDGLYQGLSTATKDTYDALHMQALPPR

SEQ ID NO: 93 - protein, 488 aa, Synthetic construct
MALPVTALLLPLALLLHAARPDIQMTQSPSSLSASVGDRVTITCKASQNVGTAVAWYQQKPGKSPKLLIFSASIRYTGVPSRFSGSGSGTDFTLTISSLQPEDFATYYCQQYSSSPYTFGGGTKVEIKGGGGSGGGGSGGGGSEVQLVQSGAEVKKPGASVKVSCKASGYTFTDYYMNWVRRAPGQRLEWMGIINPYNGGTSYNQKFRGRVTITVDKSASTAYMELSSLRSEDTAVYYCSRYDYDYDVEGAMDYWGQGTTVTVSSTTTPAPRPPTPAPTIASQPLSLRPEACRPAAGGAVHTRGLDFACDIYIWAPLAGTCGVLLLSLVITLYCKRGRKKLLYIFKQPFMRPVQTTQEEDGCSCRFPEEEEGGCELRVKFSRSADAPAYQQGQNQLYNELNLGRREEYDVLDKRRGRDPEMGGKPRRKNPQEGLYNELQKDKMAEAYSEIGMKGERRRGKGHDGLYQGLSTATKDTYDALHMQALPPR

SEQ ID NO: 94 - protein, 488 aa, Synthetic construct
MALPVTALLLPLALLLHAARPDIVMTQSPDSLAVSLGERATINCKASQNVGTAVAWYQQKPGQSPKLLIFSASIRYTGVPDRFSGSGSGTDFTLTISSLQAEDVAVYYCQQYSSSPYTFGGGTKVEIKGGGGSGGGGSGGGGSEVQLVQSGAEVKKPGASVKVSCKASGYTFTDYYMNWVRRAPGQRLEWMGIINPYNGGTSYNQKFRGRVTITVDKSASTAYMELSSLRSEDTAVYYCSRYDYDYDVEGAMDYWGQGTTVTVSSTTTPAPRPPTPAPTIASQPLSLRPEACRPAAGGAVHTRGLDFACDIYIWAPLAGTCGVLLLSLVITLYCKRGRKKLLYIFKQPFMRPVQTTQEEDGCSCRFPEEEEGGCELRVKFSRSADAPAYQQGQNQLYNELNLGRREEYDVLDKRRGRDPEMGGKPRRKNPQEGLYNELQKDKMAEAYSEIGMKGERRRGKGHDGLYQGLSTATKDTYDALHMQALPPR

SEQ ID NO: 95 - protein, 484 aa, Synthetic construct
MALPVTALLLPLALLLHAARPDIVMTQSPLSLPVTPGEPASISCRASQTISDYLHWYLQKPGQSPQLLIKYASQSISGVPDRFSGSGSGSDFTLKISRVEAEDVGVYYCQQGHSFPLTFGQGTKLEIKGGGGSGGGGSGGGGSEVQLVQSGAEVKKPGASVKVSCKASGYTFTSYWMHWVRQAPGQRLEWMGTIYPGNSDTRYNQKFKDRVTITADTSASTAYMELSSLRSEDTAVYYCTRSYDYGDLDYWGQGTTVTVSSTTTPAPRPPTPAPTIASQPLSLRPEACRPAAGGAVHTRGLDFACDIYIWAPLAGTCGVLLLSLVITLYCKRGRKKLLYIFKQPFMRPVQTTQEEDGCSCRFPEEEEGGCELRVKFSRSADAPAYQQGQNQLYNELNLGRREEYDVLDKRRGRDPEMGGKPRRKNPQEGLYNELQKDKMAEAYSEIGMKGERRRGKGHDGLYQGLSTATKDTYDALHMQALPPR

SEQ ID NO: 96 - protein, 484 aa, Synthetic construct
MALPVTALLLPLALLLHAARPDIVMTQSPLSLPVTPGEPASISCRASQTISDYLHWYLQKPGQSPRLLIKYASQSISGVPDRFSGSGSGTDFTLKISRVEAEDVGVYYCQNGHSFPLTFGQGTKLEIKGGGGSGGGGSGGGGSEVQLVQSGAEVKKPGASVKVSCKASGYTFTSYWMHWVRQAPGQRLEWMGTIYPGNSDTRYNQKFKDRVTITADTSASTAYMELSSLRSEDTAVYYCTRSYDYGDLDYWGQGTTVTVSSTTTPAPRPPTPAPTIASQPLSLRPEACRPAAGGAVHTRGLDFACDIYIWAPLAGTCGVLLLSLVITLYCKRGRKKLLYIFKQPFMRPVQTTQEEDGCSCRFPEEEEGGCELRVKFSRSADAPAYQQGQNQLYNELNLGRREEYDVLDKRRGRDPEMGGKPRRKNPQEGLYNELQKDKMAEAYSEIGMKGERRRGKGHDGLYQGLSTATKDTYDALHMQALPPR

SEQ ID NO: 97 - protein, 483 aa, Synthetic construct
MALPVTALLLPLALLLHAARPDIVMTQSPLSLPVTPGEPASISCRASQTISDYLHWYLQKPGQSPQLLIKYASQSISGVPDRFSGSGSGSDFTLKISRVEAEDVGVYYCQQGHSFPLTFGQGTKLEIKGGGGSGGGGSGGGGSEVQLVQSGAEVKKPGASVKVSCKASGYTFTSYWMHWVRQAPGQRLEWMGTIYPGNSDTRYNQKFKDRVTITADTSASTAYMELSSLRSEDTAVYYCTRSYDYGDLDYWGQGTTVTVSSAAAIEVMYPPPYLDNEKSNGTIIHVKGKHLCPSPLFPGPSKPFWVLVVVGGVLACYSLLVTVAFIIFWVRSKRSRLLHSDYMNMTPRRPGPTRKHYQPYAPPRDFAAYRSRVKFSRSADAPAYQQGQNQLYNELNLGRREEYDVLDKRRGRDPEMGGKPRRKNPQEGLYNELQKDKMAEAYSEIGMKGERRRGKGHDGLYQGLSTATKDTYDALHMQALPPR

SEQ ID NO: 98 - protein, 483 aa, Synthetic construct
MALPVTALLLPLALLLHAARPDIVMTQSPLSLPVTPGEPASISCRASQTISDYLHWYLQKPGQSPRLLIKYASQSISGVPDRFSGSGSGTDFTLKISRVEAEDVGVYYCQNGHSFPLTFGQGTKLEIKGGGGSGGGGSGGGGSEVQLVQSGAEVKKPGASVKVSCKASGYTFTSYWMHWVRQAPGQRLEWMGTIYPGNSDTRYNQKFKDRVTITADTSASTAYMELSSLRSEDTAVYYCTRSYDYGDLDYWGQGTTVTVSSAAAIEVMYPPPYLDNEKSNGTIIHVKGKHLCPSPLFPGPSKPFWVLVVVGGVLACYSLLVTVAFIIFWVRSKRSRLLHSDYMNMTPRRPGPTRKHYQPYAPPRDFAAYRSRVKFSRSADAPAYQQGQNQLYNELNLGRREEYDVLDKRRGRDPEMGGKPRRKNPQEGLYNELQKDKMAEAYSEIGMKGERRRGKGHDGLYQGLSTATKDTYDALHMQALPPR

SEQ ID NO: 99 - protein, 489 aa, Synthetic construct
MALPVTALLLPLALLLHAARPEIVLTQSPATLSLSPGERATLSCRASKSVSTSGFSYMHWYQQKPGQPPRLLIYLASNLESGIPARFSGSGSGTDFTLTISSLEPEDFAVYYCQHSRELPFTFGQGTKLEIKGGGGSGGGGSGGGGSEVQLVQSGAEVKKPGSSVKVSCKASGYAFSNYWINWVRQAPGQGLEWMGQINPGDGDTIYNSKFKGRVTITADKSTSTAYMELSSLRSEDTAVYYCEREGRNYGDFAYWGQGTTVTVSSTTTPAPRPPTPAPTIASQPLSLRPEACRPAAGGAVHTRGLDFACDIYIWAPLAGTCGVLLLSLVITLYCKRGRKKLLYIFKQPFMRPVQTTQEEDGCSCRFPEEEEGGCELRVKFSRSADAPAYQQGQNQLYNELNLGRREEYDVLDKRRGRDPEMGGKPRRKNPQEGLYNELQKDKMAEAYSEIGMKGERRRGKGHDGLYQGLSTATKDTYDALHMQALPPR

SEQ ID NO: 100 - protein, 488 aa, Synthetic construct
MALPVTALLLPLALLLHAARPEIVLTQSPATLSLSPGERATLSCRASKSVSTSGFSYMHWYQQKPGQPPRLLIYLASNLESGIPARFSGSGSGTDFTLTISSLEPEDFAVYYCQHSRELPFTFGQGTKLEIKGGGGSGGGGSGGGGSEVQLVQSGAEVKKPGSSVKVSCKASGYAFSNYWINWVRQAPGQGLEWMGQINPGDGDTIYNSKFKGRVTITADKSTSTAYMELSSLRSEDTAVYYCEREGRNYGDFAYWGQGTTVTVSSAAAIEVMYPPPYLDNEKSNGTIIHVKGKHLCPSPLFPGPSKPFWVLVVVGGVLACYSLLVTVAFIIFWVRSKRSRLLHSDYMNMTPRRPGPTRKHYQPYAPPRDFAAYRSRVKFSRSADAPAYQQGQNQLYNELNLGRREEYDVLDKRRGRDPEMGGKPRRKNPQEGLYNELQKDKMAEAYSEIGMKGERRRGKGHDGLYQGLSTATKDTYDALHMQALPPR

SEQ ID NO: 101 - protein, 17 aa, Synthetic construct
IINPYNSGTSYNQKFRG

SEQ ID NO: 102 - protein, 155 aa, Synthetic construct
QRFAQAQQQLPLESLGWDVAELQLNHTGPQQDPRLYWQGGPALGRSFLHGPELDKGQLRIHRDGIYMVHIQVTLAICSSTTASRHHPTTLAVGICSPASRSISLLRLSFHQGCTIASQRLTPLARGDTLCTNLTGTLLPSRNTDETFFGVQWVRP

SEQ ID NO: 103 - protein, 686 aa, Synthetic construct
MALPVTALLLPLALLLHAARPDIVMTQSPLSLPVTPGEPASISCRASQTISDYLHWYLQKPGQSPQLLIKYASQSISGVPDRFSGSGSGSDFTLKISRVEAEDVGVYYCQQGHSFPLTFGQGTKLEIKGGGGSGGGGSGGGGSEVQLVQSGAEVKKPGASVKVSCKASGYTFTSYWMHWVRQAPGQRLEWMGTIYPGNSDTRYNQKFKDRVTITADTSASTAYMELSSLRSEDTAVYYCTRSYDYGDLDYWGQGTTVTVSSTTTPAPRPPTPAPTIASQPLSLRPEACRPAAGGAVHTRGLDFACDIYIWAPLAGTCGVLLLSLVITLYCKRGRKKLLYIFKQPFMRPVQTTQEEDGCSCRFPEEEEGGCELRVKFSRSADAPAYQQGQNQLYNELNLGRREEYDVLDKRRGRDPEMGGKPRRKNPQEGLYNELQKDKMAEAYSEIGMKGERRRGKGHDGLYQGLSTATKDTYDALHMQALPPRKRRSGSGATNFSLLKQAGDVEENPGPMALPVTALLLPLALLLHAARPQRFAQAQQQLPLESLGWDVAELQLNHTGPQQDPRLYWQGGPALGRSFLHGPELDKGQLRIHRDGIYMVHIQVTLAICSSTTASRHHPTTLAVGICSPASRSISLLRLSFHQGCTIASQRLTPLARGDTLCTNLTGTLLPSRNTDETFFGVQWVRP

SEQ ID NO: 104 - protein, 193 aa, Synthetic construct
MPEEGSGCSVRRRPYGCVLRAALVPLVAGLVICLVVCIQRFAQAQQQLPLESLGWDVAELQLNHTGPQQDPRLYWQGGPALGRSFLHGPELDKGQLRIHRDGIYMVHIQVTLAICSSTTASRHHPTTLAVGICSPASRSISLLRLSFHQGCTIASQRLTPLARGDTLCTNLTGTLLPSRNTDETFFGVQWVRP

SEQ ID NO: 105 - protein, 703 aa, Synthetic construct
MALPVTALLLPLALLLHAARPDIVMTQSPLSLPVTPGEPASISCRASQTISDYLHWYLQKPGQSPQLLIKYASQSISGVPDRFSGSGSGSDFTLKISRVEAEDVGVYYCQQGHSFPLTFGQGTKLEIKGGGGSGGGGSGGGGSEVQLVQSGAEVKKPGASVKVSCKASGYTFTSYWMHWVRQAPGQRLEWMGTIYPGNSDTRYNQKFKDRVTITADTSASTAYMELSSLRSEDTAVYYCTRSYDYGDLDYWGQGTTVTVSSTTTPAPRPPTPAPTIASQPLSLRPEACRPAAGGAVHTRGLDFACDIYIWAPLAGTCGVLLLSLVITLYCKRGRKKLLYIFKQPFMRPVQTTQEEDGCSCRFPEEEEGGCELRVKFSRSADAPAYQQGQNQLYNELNLGRREEYDVLDKRRGRDPEMGGKPRRKNPQEGLYNELQKDKMAEAYSEIGMKGERRRGKGHDGLYQGLSTATKDTYDALHMQALPPRKRRSGSGATNFSLLKQAGDVEENPGPMPEEGSGCSVRRRPYGCVLRAALVPLVAGLVICLVVCIQRFAQAQQQLPLESLGWDVAELQLNHTGPQQDPRLYWQGGPALGRSFLHGPELDKGQLRIHRDGIYMVHIQVTLAICSSTTASRHHPTTLAVGICSPASRSISLLRLSFHQGCTIASQRLTPLARGDTLCTNLTGTLLPSRNTDETFFGVQWVRP

SEQ ID NO: 106 - protein, 19 aa, Synthetic construct
ATNFSLLKQAGDVEENPGP